European Patent Application EP 4 649 966 A2, published November 19, 2025. Title: RADIOLABELED ANTI-PD-L1 ANTIBODIES FOR IMMUNO-PET IMAGING. Applicant: REGENERON PHARMACEUTICALS, INC. The sequence listing filed with the application follows.

SEQUENCE LISTING (344 sequences)

SEQ ID NO: 1 - DNA, 363 bp, synthetic construct
  misc_feature 1..363: note = synthetic
  source 1..363: mol_type = other DNA
gaggtgcagctggtggagtctgggggaggcttggtccagcctggggggtccctgagactctcctgtgcagcctctggattcacctttagtaggttttggatgagctgggtccgccaggctccagggaaggggctggagtgggtggccaacataaaccaagatggaactgagaaatactatgtggactctgtgaagggccgattcaccatctccagagacaacgccaagaactcactgtatctgcaaatgaacagcctgagagccggggacacggctgtgtattactgtgcgaatacgtattacgatttttggagtggtcactttgactactggggccagggaaccctggtcaccgtctcctca

SEQ ID NO: 2 - protein, 121 aa, synthetic construct
  REGION 1..121: note = synthetic
EVQLVESGGGLVQPGGSLRLSCAASGFTFSRFWMSWVRQAPGKGLEWVANINQDGTEKYYVDSVKGRFTISRDNAKNSLYLQMNSLRAGDTAVYYCANTYYDFWSGHFDYWGQGTLVTVSS

SEQ ID NO: 3 - DNA, 24 bp, synthetic construct
  misc_feature 1..24: note = synthetic
  source 1..24: mol_type = other DNA
ggattcacctttagtaggttttgg

SEQ ID NO: 4 - protein, 8 aa, synthetic construct
  REGION 1..8: note = synthetic
GFTFSRFW

SEQ ID NO: 5 - DNA, 24 bp, synthetic construct
  misc_feature 1..24: note = synthetic
  source 1..24: mol_type = other DNA
ataaaccaagatggaactgagaaa

SEQ ID NO: 6 - protein, 8 aa, synthetic construct
  REGION 1..8: note = synthetic
INQDGTEK

SEQ ID NO: 7 - DNA, 42 bp, synthetic construct
  misc_feature 1..42: note = synthetic
  source 1..42: mol_type = other DNA
gcgaatacgtattacgatttttggagtggtcactttgactac

SEQ ID NO: 8 - protein, 14 aa, synthetic construct
  REGION 1..14: note = synthetic
ANTYYDFWSGHFDY

SEQ ID NO: 9 - DNA, 321 bp, synthetic construct
  misc_feature 1..321: note = synthetic
  source 1..321: mol_type = other DNA
gacatccagatgacccagtctccttccaccctgtctgcatctgtaggagacagagtcaccatcacttgtcgggccagtcagagtattagtaattggttggcctggtatcagcagaaaccagggaaagcccctaagctcctgatctataaggcgtctagtttagaaagtggggtcccatcaaggttcagcggcagtggatctgggacagaattcactctcaccatcagcagcctgcagcctgatgattttgcaacttattactgccaacagtatcatagttattcgtacacttttggccaggggaccaagctggagatcaaa

SEQ ID NO: 10 - protein, 107 aa, synthetic construct
  REGION 1..107: note = synthetic
DIQMTQSPSTLSASVGDRVTITCRASQSISNWLAWYQQKPGKAPKLLIYKASSLESGVPSRFSGSGSGTEFTLTISSLQPDDFATYYCQQYHSYSYTFGQGTKLEIK

SEQ ID NO: 11 - DNA, 18 bp, synthetic construct
  misc_feature 1..18: note = synthetic
  source 1..18: mol_type = other DNA
cagagtattagtaattgg

SEQ ID NO: 12 - protein, 6 aa, synthetic construct
  REGION 1..6: note = synthetic
QSISNW

SEQ ID NO: 13-14 - skipped (2 entries)

SEQ ID NO: 15 - DNA, 27 bp, synthetic construct
  misc_feature 1..27: note = synthetic
  source 1..27: mol_type = other DNA
caacagtatcatagttattcgtacact

SEQ ID NO: 16 - protein, 9 aa, synthetic construct
  REGION 1..9: note = synthetic
QQYHSYSYT

SEQ ID NO: 17 - DNA, 363 bp, synthetic construct
  misc_feature 1..363: note = synthetic
  source 1..363: mol_type = other DNA
caggagcacctggtggagtctgggggaggcgtggtccagcctgggaggtccctgagactctcctgtgaagcgtctggattcaccttcagtaactttggcatgcactgggtccgccaggctccaggcaaggggctggagtgggtggcagctttatggtctgatggaagtaataaatactatgcagactccgtgaagggtcgagtcaccatctccagagacaattccaagaacacactgtatctgcaaatgaacagcctgagagccgaggacacggctgtctattactgtgcgagagggagaggagcccccggtattccgatttttgggtactggggccagggaaccctggtcaccgtctcctca

SEQ ID NO: 18 - protein, 121 aa, synthetic construct
  REGION 1..121: note = synthetic
QEHLVESGGGVVQPGRSLRLSCEASGFTFSNFGMHWVRQAPGKGLEWVAALWSDGSNKYYADSVKGRVTISRDNSKNTLYLQMNSLRAEDTAVYYCARGRGAPGIPIFGYWGQGTLVTVSS

SEQ ID NO: 19 - DNA, 24 bp, synthetic construct
  misc_feature 1..24: note = synthetic
  source 1..24: mol_type = other DNA
ggattcaccttcagtaactttggc

SEQ ID NO: 20 - protein, 8 aa, synthetic construct
  REGION 1..8: note = synthetic
GFTFSNFG

SEQ ID NO: 21 - DNA, 24 bp, synthetic construct
  misc_feature 1..24: note = synthetic
  source 1..24: mol_type = other DNA
ttatggtctgatggaagtaataaa

SEQ ID NO: 22 - protein, 8 aa, synthetic construct
  REGION 1..8: note = synthetic
LWSDGSNK

SEQ ID NO: 23 - DNA, 42 bp, synthetic construct
  misc_feature 1..42: note = synthetic
  source 1..42: mol_type = other DNA
gcgagagggagaggagcccccggtattccgatttttgggtac

SEQ ID NO: 24 - protein, 14 aa, synthetic construct
  REGION 1..14: note = synthetic
ARGRGAPGIPIFGY

SEQ ID NO: 25 - DNA, 321 bp, synthetic construct
  misc_feature 1..321: note = synthetic
  source 1..321: mol_type = other DNA
gacatccagatgacccagtctccatcctccctgtctgcatctgttggagacagagtcaccatcacttgccgggcaagtcagggcattagaaatgatttaggctggtatcagcagaaaccagggaaagcccctaagcgcctgatctatactgcatccagtttgcaaagtggggtcccatcaagattcagcggcagtggatctgggacagaattcactctcacaatcagcagcctacagcctgaagattttgcaacttattactgtctacaacataatagttaccctctcacattcggcggagggaccaaggtggcgatcaaa

SEQ ID NO: 26 - protein, 107 aa, synthetic construct
  REGION 1..107: note = synthetic
DIQMTQSPSSLSASVGDRVTITCRASQGIRNDLGWYQQKPGKAPKRLIYTASSLQSGVPSRFSGSGSGTEFTLTISSLQPEDFATYYCLQHNSYPLTFGGGTKVAIK

SEQ ID NO: 27 - DNA, 18 bp, synthetic construct
  misc_feature 1..18: note = synthetic
  source 1..18: mol_type = other DNA
cagggcattagaaatgat

SEQ ID NO: 28 - protein, 6 aa, synthetic construct
  REGION 1..6: note = synthetic
QGIRND

SEQ ID NO: 29-30 - skipped (2 entries)

SEQ ID NO: 31 - DNA, 27 bp, synthetic construct
  misc_feature 1..27: note = synthetic
  source 1..27: mol_type = other DNA
ctacaacataatagttaccctctcaca

SEQ ID NO: 32 - protein, 9 aa, synthetic construct
  REGION 1..9: note = synthetic
LQHNSYPLT

SEQ ID NO: 33 - DNA, 390 bp, synthetic construct
  misc_feature 1..390: note = synthetic
  source 1..390: mol_type = other DNA
gaggtgcagctggtggagtctgggggaggcttggtaaagcctggggggtcccttagactctcctgtgcagcctctggattcactttcagtaacgcctggatgagctgggtccgccaggctccagggaaggggctggagtgggttggccgtattaaaaggaaaactgatggtgggacaacagactacgctgcacccgtgaaaggcagattcaccatctcaagagatgattcaaaaaatacgctgcatctgcaaatgaacagcctgaaaaccgaggacacagccgtgtattactgtaccacagatgatattgtagttgtaccagctgttatgagggaatactacttcggtatggacgtctggggccaagggaccacggtcaccgtctcctca

SEQ ID NO: 34 - protein, 130 aa, synthetic construct
  REGION 1..130: note = synthetic
EVQLVESGGGLVKPGGSLRLSCAASGFTFSNAWMSWVRQAPGKGLEWVGRIKRKTDGGTTDYAAPVKGRFTISRDDSKNTLHLQMNSLKTEDTAVYYCTTDDIVVVPAVMREYYFGMDVWGQGTTVTVSS

SEQ ID NO: 35 - DNA, 24 bp, synthetic construct
  misc_feature 1..24: note = synthetic
  source 1..24: mol_type = other DNA
ggattcactttcagtaacgcctgg

SEQ ID NO: 36 - protein, 8 aa, synthetic construct
  REGION 1..8: note = synthetic
GFTFSNAW

SEQ ID NO: 37 - DNA, 30 bp, synthetic construct
  misc_feature 1..30: note = synthetic
  source 1..30: mol_type = other DNA
attaaaaggaaaactgatggtgggacaaca

SEQ ID NO: 38 - protein, 10 aa, synthetic construct
  REGION 1..10: note = synthetic
IKRKTDGGTT

SEQ ID NO: 39 - DNA, 63 bp, synthetic construct
  misc_feature 1..63: note = synthetic
  source 1..63: mol_type = other DNA
accacagatgatattgtagttgtaccagctgttatgagggaatactacttcggtatggacgtc

SEQ ID NO: 40 - protein, 21 aa, synthetic construct
  REGION 1..21: note = synthetic
TTDDIVVVPAVMREYYFGMDV

SEQ ID NO: 41 - DNA, 321 bp, synthetic construct
  misc_feature 1..321: note = synthetic
  source 1..321: mol_type = other DNA
gacatccagatgacccagtctccatcctccctgtctgcatctgtaggagacagagtcaccatcacttgccggacaagtcagggcattagaaatgatttaggctggtatcagcagaaaccagggaaagcccctaagcgcctgatctatgctgcatccagtttgcaaagtggggtcccatcaaggttcagcggcagtggatctgggacagaattcactctcacaatcagcagcctgcagcctgaagattttgcaacttattactgtctacagcataataattacccgtacacttttggccaggggaccaagctggagatcaaa

SEQ ID NO: 42 - protein, 107 aa, synthetic construct
  REGION 1..107: note = synthetic
DIQMTQSPSSLSASVGDRVTITCRTSQGIRNDLGWYQQKPGKAPKRLIYAASSLQSGVPSRFSGSGSGTEFTLTISSLQPEDFATYYCLQHNNYPYTFGQGTKLEIK

SEQ ID NO: 43 - DNA, 18 bp, synthetic construct
  misc_feature 1..18: note = synthetic
  source 1..18: mol_type = other DNA
cagggcattagaaatgat

SEQ ID NO: 44 - protein, 6 aa, synthetic construct
  REGION 1..6: note = synthetic
QGIRND

SEQ ID NO: 45-46 - skipped (2 entries)

SEQ ID NO: 47 - DNA, 27 bp, synthetic construct
  misc_feature 1..27: note = synthetic
  source 1..27: mol_type = other DNA
ctacagcataataattacccgtacact

SEQ ID NO: 48 - protein, 9 aa, synthetic construct
  REGION 1..9: note = synthetic
LQHNNYPYT

SEQ ID NO: 49 - DNA, 363 bp, synthetic construct
  misc_feature 1..363: note = synthetic
  source 1..363: mol_type = other DNA
caggtgcaattggtgcagtctggggcggaggtgaagaagcctggggcctcagtgcaggtctcctgcaaggcttctggatactccttcaccggctactatatacactgggtgcgacaggcccctggacaaggacttgagtggatgggatggatcaaccctaacagtggcaccaaaaagtatgcacacaagtttcagggcagggtcaccatgaccagggacacgtccatcgacacagcctacatgattttgagcagtctgatatccgacgacacggccgtgtattactgtgcgagagatgaggactggaactttgggagctggttcgactcctggggccagggaaccctggtcaccgtctcctca

SEQ ID NO: 50 - protein, 121 aa, synthetic construct
  REGION 1..121: note = synthetic
QVQLVQSGAEVKKPGASVQVSCKASGYSFTGYYIHWVRQAPGQGLEWMGWINPNSGTKKYAHKFQGRVTMTRDTSIDTAYMILSSLISDDTAVYYCARDEDWNFGSWFDSWGQGTLVTVSS

SEQ ID NO: 51 - DNA, 24 bp, synthetic construct
  misc_feature 1..24: note = synthetic
  source 1..24: mol_type = other DNA
ggatactccttcaccggctactat

SEQ ID NO: 52 - protein, 8 aa, synthetic construct
  REGION 1..8: note = synthetic
GYSFTGYY

SEQ ID NO: 53 - DNA, 24 bp, synthetic construct
  misc_feature 1..24: note = synthetic
  source 1..24: mol_type = other DNA
atcaaccctaacagtggcaccaaa

SEQ ID NO: 54 - protein, 8 aa, synthetic construct
  REGION 1..8: note = synthetic
INPNSGTK

SEQ ID NO: 55 - DNA, 42 bp, synthetic construct
  misc_feature 1..42: note = synthetic
  source 1..42: mol_type = other DNA
gcgagagatgaggactggaactttgggagctggttcgactcc

SEQ ID NO: 56 - protein, 14 aa, synthetic construct
  REGION 1..14: note = synthetic
ARDEDWNFGSWFDS

SEQ ID NO: 57 - DNA, 336 bp, synthetic construct
  misc_feature 1..336: note = synthetic
  source 1..336: mol_type = other DNA
gatattgtgatgacccagactccactctcctcacctgtcacccttggacagccggcctccatctcctgcaggtctagtcaaaccctcgtacacggtgatggaaacacgtacttgagttggattcagcagaggccaggccagcctccgagactcctcatttataaggtttctaatcagttctctggggtcccagacagattcagtggcagtggggcagggacagatttcacactgaaaatcagcagggtggaagctgaggatgtcgggctttatttctgcatgcaagctacacattttccgatcaccttcggccaagggacacgactggagattaaa

SEQ ID NO: 58 - protein, 112 aa, synthetic construct
  REGION 1..112: note = synthetic
DIVMTQTPLSSPVTLGQPASISCRSSQTLVHGDGNTYLSWIQQRPGQPPRLLIYKVSNQFSGVPDRFSGSGAGTDFTLKISRVEAEDVGLYFCMQATHFPITFGQGTRLEIK

SEQ ID NO: 59 - DNA, 33 bp, synthetic construct
  misc_feature 1..33: note = synthetic
  source 1..33: mol_type = other DNA
caaaccctcgtacacggtgatggaaacacgtac

SEQ ID NO: 60 - protein, 11 aa, synthetic construct
  REGION 1..11: note = synthetic
QTLVHGDGNTY

SEQ ID NO: 61-62 - skipped (2 entries)

SEQ ID NO: 63 - DNA, 27 bp, synthetic construct
  misc_feature 1..27: note = synthetic
  source 1..27: mol_type = other DNA
atgcaagctacacattttccgatcacc

SEQ ID NO: 64 - protein, 9 aa, synthetic construct
  REGION 1..9: note = synthetic
MQATHFPIT

SEQ ID NO: 65 - DNA, 363 bp, synthetic construct
  misc_feature 1..363: note = synthetic
  source 1..363: mol_type = other DNA
caggtacacctggtgcagtctggggctgaggtgaagaagcctggggcctcagtgaaggtctcctgcaaggcttctggatacaccttcaccggctactatatacattgggtgcgacaggcccctggacacgggcttgagtggatgggatggctcaaccctaatactggtaccacaaagtatatacagaactttcagggcagggtcaccatgaccagggacacgtccagcagcacagcctacatggagctgaccaggctgagatctgacgacacggccgtgtattactgtgcgagagatgaggactggaattatgggagctggttcgacacctggggccagggaaccctggtcacagtctcctca

SEQ ID NO: 66 - protein, 121 aa, synthetic construct
  REGION 1..121: note = synthetic
QVHLVQSGAEVKKPGASVKVSCKASGYTFTGYYIHWVRQAPGHGLEWMGWLNPNTGTTKYIQNFQGRVTMTRDTSSSTAYMELTRLRSDDTAVYYCARDEDWNYGSWFDTWGQGTLVTVSS

SEQ ID NO: 67 - DNA, 24 bp, synthetic construct
  misc_feature 1..24: note = synthetic
  source 1..24: mol_type = other DNA
ggatacaccttcaccggctactat

SEQ ID NO: 68 - protein, 8 aa, synthetic construct
  REGION 1..8: note = synthetic
GYTFTGYY

SEQ ID NO: 69 - DNA, 24 bp, synthetic construct
  misc_feature 1..24: note = synthetic
  source 1..24: mol_type = other DNA
ctcaaccctaatactggtaccaca

SEQ ID NO: 70 - protein, 8 aa, synthetic construct
  REGION 1..8: note = synthetic
LNPNTGTT

SEQ ID NO: 71 - DNA, 42 bp, synthetic construct
  misc_feature 1..42: note = synthetic
  source 1..42: mol_type = other DNA
gcgagagatgaggactggaattatgggagctggttcgacacc

SEQ ID NO: 72 - protein, 14 aa, synthetic construct
  REGION 1..14: note = synthetic
ARDEDWNYGSWFDT

SEQ ID NO: 73 - DNA, 336 bp, synthetic construct
  misc_feature 1..336: note = synthetic
  source 1..336: mol_type = other DNA
gatattgtaatgacccagactccactctcctcacctgtcacccttggacagccggcctccatctcctgcaggtctagtccaagcctcgtacacagtgatggaaacacctacttgagttggcttcagcagaggccaggccagcctccaagactcctaatttataagatttctaaccgattctctggggtcccagacagattcagtggcagtggggcagggacagatttcacgctgaaaatcagcagggtggaagctgaggatgtcggggtttattactgcatgcaagctacacattttccgatcaccttcggccaagggacacgactggagattaga

SEQ ID NO: 74 - protein, 112 aa, synthetic construct
  REGION 1..112: note = synthetic
DIVMTQTPLSSPVTLGQPASISCRSSPSLVHSDGNTYLSWLQQRPGQPPRLLIYKISNRFSGVPDRFSGSGAGTDFTLKISRVEAEDVGVYYCMQATHFPITFGQGTRLEIR

SEQ ID NO: 75 - DNA, 33 bp, synthetic construct
  misc_feature 1..33: note = synthetic
  source 1..33: mol_type = other DNA
ccaagcctcgtacacagtgatggaaacacctac

SEQ ID NO: 76 - protein, 11 aa, synthetic construct
  REGION 1..11: note = synthetic
PSLVHSDGNTY

SEQ ID NO: 77-78 - skipped (2 entries)

SEQ ID NO: 79 - DNA, 27 bp, synthetic construct
  misc_feature 1..27: note = synthetic
  source 1..27: mol_type = other DNA
atgcaagctacacattttccgatcacc

SEQ ID NO: 80 - protein, 9 aa, synthetic construct
  REGION 1..9: note = synthetic
MQATHFPIT

SEQ ID NO: 81 - DNA, 360 bp, synthetic construct
  misc_feature 1..360: note = synthetic
  source 1..360: mol_type = other DNA
gaggtgcagctggtggaatctgggggaggtgtggtgcggcctggggggtccctgagactctcctgtgcagcctctggattcacttttgatgattatggcatgacctgggtccgccaagctccagggaggggcctggaatgggtctctggtattcattggcatggtaaacgcacaggttatgcagactctgtgaagggccgattcaccatatccagagacaacgccaagaaatccctgtatctgcaaatgaacagtctgaaaggcgaggacacggccttgtatcattgtgtgagggggggaatgagtacaggggactggttcgacccctggggccagggaaccctggtcatcgtctcctca

SEQ ID NO: 82 - protein, 120 aa, synthetic construct
  REGION 1..120: note = synthetic
EVQLVESGGGVVRPGGSLRLSCAASGFTFDDYGMTWVRQAPGRGLEWVSGIHWHGKRTGYADSVKGRFTISRDNAKKSLYLQMNSLKGEDTALYHCVRGGMSTGDWFDPWGQGTLVIVSS

SEQ ID NO: 83 - DNA, 24 bp, synthetic construct
  misc_feature 1..24: note = synthetic
  source 1..24: mol_type = other DNA
ggattcacttttgatgattatggc

SEQ ID NO: 84 - protein, 8 aa, synthetic construct
  REGION 1..8: note = synthetic
GFTFDDYG

SEQ ID NO: 85 - DNA, 24 bp, synthetic construct
  misc_feature 1..24: note = synthetic
  source 1..24: mol_type = other DNA
attcattggcatggtaaacgcaca

SEQ ID NO: 86 - protein, 8 aa, synthetic construct
  REGION 1..8: note = synthetic
IHWHGKRT

SEQ ID NO: 87 - DNA, 39 bp, synthetic construct
  misc_feature 1..39: note = synthetic
  source 1..39: mol_type = other DNA
gtgagggggggaatgagtacaggggactggttcgacccc

SEQ ID NO: 88 - protein, 13 aa, synthetic construct
  REGION 1..13: note = synthetic
VRGGMSTGDWFDP

SEQ ID NO: 89 - DNA, 324 bp, synthetic construct
  misc_feature 1..324: note = synthetic
  source 1..324: mol_type = other DNA
gacatccagatgacccagtctccatcctccctgtctgcatctctaggagacagagtcaccatcacttgccgggcaagtcagagcattaacagttatttaaattggtatcagcagaaaccagggaaagcccctaaactcctgatctatgttgcatccagtttgcaaagtggggtcccatcaaggttcagtggcagtggatctgggacagaattcactctcaccatcagcaatctgcaacctgaagattttgcaacttactactgtcaacagagttacagtacccctccgatcaccttcggccaagggacacgactggagattaaa

SEQ ID NO: 90 - protein, 108 aa, synthetic construct
  REGION 1..108: note = synthetic
DIQMTQSPSSLSASLGDRVTITCRASQSINSYLNWYQQKPGKAPKLLIYVASSLQSGVPSRFSGSGSGTEFTLTISNLQPEDFATYYCQQSYSTPPITFGQGTRLEIK

SEQ ID NO: 91 - DNA, 18 bp, synthetic construct
  misc_feature 1..18: note = synthetic
  source 1..18: mol_type = other DNA
cagagcattaacagttat

SEQ ID NO: 92 - protein, 6 aa, synthetic construct
  REGION 1..6: note = synthetic
QSINSY

SEQ ID NO: 93-94 - skipped (2 entries)

SEQ ID NO: 95 - DNA, 30 bp, synthetic construct
  misc_feature 1..30: note = synthetic
  source 1..30: mol_type = other DNA
caacagagttacagtacccctccgatcacc

SEQ ID NO: 96 - protein, 10 aa, synthetic construct
  REGION 1..10: note = synthetic
QQSYSTPPIT

SEQ ID NO: 97 - DNA, 360 bp, synthetic construct
  misc_feature 1..360: note = synthetic
  source 1..360: mol_type = other DNA
gaggtgcagctggtggagtctgggggaggtgtggtacggccgggggggtccctgagactctcctgtgcagcctctggattcacctttgatgattatggcatgacctgggtccgccaagttccagggaaggggctggagtgggtctctggtattcattggagtggtagaagcacaggttatgcagactctgtgaagggccgattcaccatctccagagacaacgccaagaactccctgtatctgcaaatgaacagtctgagagccgaggacacggccttgtattactgtgcgagggggggaatgagtacgggggactggttcgacccctggggccagggaaccctggtcaccgtctcctca

SEQ ID NO: 98 - protein, 120 aa, synthetic construct
  REGION 1..120: note = synthetic
EVQLVESGGGVVRPGGSLRLSCAASGFTFDDYGMTWVRQVPGKGLEWVSGIHWSGRSTGYADSVKGRFTISRDNAKNSLYLQMNSLRAEDTALYYCARGGMSTGDWFDPWGQGTLVTVSS

SEQ ID NO: 99 - DNA, 24 bp, synthetic construct
  misc_feature 1..24: note = synthetic
  source 1..24: mol_type = other DNA
ggattcacctttgatgattatggc

SEQ ID NO: 100 - protein, 8 aa, synthetic construct
  REGION 1..8: note = synthetic
GFTFDDYG

SEQ ID NO: 101 - DNA, 24 bp, synthetic construct
  misc_feature 1..24: note = synthetic
  source 1..24: mol_type = other DNA
attcattggagtggtagaagcaca

SEQ ID NO: 102 - protein, 8 aa, synthetic construct
  REGION 1..8: note = synthetic
IHWSGRST

SEQ ID NO: 103 - DNA, 39 bp, synthetic construct
  misc_feature 1..39: note = synthetic
  source 1..39: mol_type = other DNA
gcgagggggggaatgagtacgggggactggttcgacccc

SEQ ID NO: 104 - protein, 13 aa, synthetic construct
  REGION 1..13: note = synthetic
ARGGMSTGDWFDP

SEQ ID NO: 105 - DNA, 324 bp, synthetic construct
  misc_feature 1..324: note = synthetic
  source 1..324: mol_type = other DNA
gacatccagatgacccagtctccatcctccctgtctgcatctgtaggagacagagtcaccatcacttgccgggcaagtcagagcattagcagctatttaaattggtatcagcagaaaccagggaaagcccctaagctcctgatctatgttgcatccagtttgcaaagtggggtcccatcaaggttcagtggcagtggatctgggacagatttcactctcaccatcagcagtctgcaacctgaagattttgcaacttactactgtcaacagagttacagtacccctccgatcaccttcggccaagggacacgactggagattaaa

SEQ ID NO: 106 - protein, 108 aa, synthetic construct
  REGION 1..108: note = synthetic
DIQMTQSPSSLSASVGDRVTITCRASQSISSYLNWYQQKPGKAPKLLIYVASSLQSGVPSRFSGSGSGTDFTLTISSLQPEDFATYYCQQSYSTPPITFGQGTRLEIK

SEQ ID NO: 107 - DNA, 18 bp, synthetic construct
  misc_feature 1..18: note = synthetic
  source 1..18: mol_type = other DNA
cagagcattagcagctat

SEQ ID NO: 108 - protein, 6 aa, synthetic construct
  REGION 1..6: note = synthetic
QSISSY

SEQ ID NO: 109-110 - skipped (2 entries)

SEQ ID NO: 111 - DNA, 30 bp, synthetic construct; identical to SEQ ID NO: 95
  misc_feature 1..30: note = synthetic
  source 1..30: mol_type = other DNA

SEQ ID NO: 112 - protein, 10 aa, synthetic construct
  REGION 1..10: note = synthetic
QQSYSTPPIT

SEQ ID NO: 113 - DNA, 345 bp, synthetic construct
  misc_feature 1..345: note = synthetic
  source 1..345: mol_type = other DNA
gaggtgcagttggtggagtctggaggaggcttggtccagcctggggggtccctaagactctcctgtgcagcctctgggttcaccgtcggtagtaactacatgaactgggtccgtcaggctccagggaagggactggagtgggtctcagttatttatagtggtggtagtacatactacgcagattccgtgaagggccgattcaccatctccagactcacttccaagaacacactgtatcttcaaatgagcagcctgagacctgaggacacggccgtgtattattgtgcgagagggattaggggtctggacgtctggggccaagggaccacggtcaccgtctcttca

SEQ ID NO: 114 - protein, 115 aa, synthetic construct
  REGION 1..115: note = synthetic
EVQLVESGGGLVQPGGSLRLSCAASGFTVGSNYMNWVRQAPGKGLEWVSVIYSGGSTYYADSVKGRFTISRLTSKNTLYLQMSSLRPEDTAVYYCARGIRGLDVWGQGTTVTVSS

SEQ ID NO: 115 - DNA, 24 bp, synthetic construct
  misc_feature 1..24: note = synthetic
  source 1..24: mol_type = other DNA
gggttcaccgtcggtagtaactac

SEQ ID NO: 116 - protein, 8 aa, synthetic construct
  REGION 1..8: note = synthetic
GFTVGSNY

SEQ ID NO: 117 - DNA, 21 bp, synthetic construct
  misc_feature 1..21: note = synthetic
  source 1..21: mol_type = other DNA
atttatagtggtggtagtaca

SEQ ID NO: 118 - protein, 7 aa, synthetic construct
  REGION 1..7: note = synthetic
IYSGGST

SEQ ID NO: 119 - DNA, 27 bp, synthetic construct
  misc_feature 1..27: note = synthetic
  source 1..27: mol_type = other DNA
gcgagagggattaggggtctggacgtc

SEQ ID NO: 120 - protein, 9 aa, synthetic construct
  REGION 1..9: note = synthetic
ARGIRGLDV

SEQ ID NO: 121 - DNA, 324 bp, synthetic construct
  misc_feature 1..324: note = synthetic
  source 1..324: mol_type = other DNA
gacatccagatgacccagtctccatcctccctgtctgcatctgtaggagacagagtcaccatcacttgccgggcaagtcagaccattaacatctatttaaattggtatcagcagaaaccagggagagcccctaggctcctgatctatgctgcatccagtttgcaaagtggggtcccatcaaggttcagtggcagtggatctgggacagatttcactctcaccatcagcagtctgcaacctgaagattttgcaacttactactgtcaccagagttacagtacccctccgatcaccttcggccaagggacacgactggagattaaa

SEQ ID NO: 122 - protein, 108 aa, synthetic construct
  REGION 1..108: note = synthetic
DIQMTQSPSSLSASVGDRVTITCRASQTINIYLNWYQQKPGRAPRLLIYAASSLQSGVPSRFSGSGSGTDFTLTISSLQPEDFATYYCHQSYSTPPITFGQGTRLEIK

SEQ ID NO: 123 - DNA, 18 bp, synthetic construct
  misc_feature 1..18: note = synthetic
  source 1..18: mol_type = other DNA
cagaccattaacatctat

SEQ ID NO: 124 - protein, 6 aa, synthetic construct
  REGION 1..6: note = synthetic
QTINIY

SEQ ID NO: 125-126 - skipped (2 entries)

SEQ ID NO: 127 - DNA, 30 bp, synthetic construct
  misc_feature 1..30: note = synthetic
  source 1..30: mol_type = other DNA
caccagagttacagtacccctccgatcacc

SEQ ID NO: 128 - protein, 10 aa, synthetic construct
  REGION 1..10: note = synthetic
HQSYSTPPIT

SEQ ID NO: 129 - DNA, 345 bp, synthetic construct
  misc_feature 1..345: note = synthetic
  source 1..345: mol_type = other DNA
gaggaacggttggtggagtctggaggagacttggtccagcctggggggtccctgagactctcctgtgcagcctctggcatcaccgtcggtactaattatatgaactgggtccgccaggctccagggaagggactggagtgggtctcagttatttctagcggtggtaatacacactacgcagactccgtgaagggccgattcattatgtccagacaaacttccaaaaacacgctgtatcttcagatgaatagcctggaaactgaggacacggccgtatattattgtgcgagggggatcagaggtttggacgtctggggccaagggaccatggtcaccgtctcctca

SEQ ID NO: 130 - protein, 115 aa, synthetic construct
  REGION 1..115: note = synthetic
EERLVESGGDLVQPGGSLRLSCAASGITVGTNYMNWVRQAPGKGLEWVSVISSGGNTHYADSVKGRFIMSRQTSKNTLYLQMNSLETEDTAVYYCARGIRGLDVWGQGTMVTVSS

SEQ ID NO: 131 - DNA, 24 bp, synthetic construct
  misc_feature 1..24: note = synthetic
  source 1..24: mol_type = other DNA
ggcatcaccgtcggtactaattat

SEQ ID NO: 132 - protein, 8 aa, synthetic construct
  REGION 1..8: note = synthetic
GITVGTNY

SEQ ID NO: 133 - DNA, 21 bp, synthetic construct
  misc_feature 1..21: note = synthetic
  source 1..21: mol_type = other DNA
atttctagcggtggtaataca

SEQ ID NO: 134 - protein, 7 aa, synthetic construct
  REGION 1..7: note = synthetic
ISSGGNT

SEQ ID NO: 135 - DNA, 27 bp, synthetic construct
  misc_feature 1..27: note = synthetic
  source 1..27: mol_type = other DNA
gcgagggggatcagaggtttggacgtc

SEQ ID NO: 136 - protein, 9 aa, synthetic construct
  REGION 1..9: note = synthetic
ARGIRGLDV

SEQ ID NO: 137 - DNA, 324 bp, synthetic construct
  misc_feature 1..324: note = synthetic
  source 1..324: mol_type = other DNA
gacatccagatgacccagtctccatcctccctgtctgcatctgtaggagacagagtcaccatcacttgccgggcaagtcagagcatgagcagctatttaaattggtatcagcagaaaccagggagagcccctaagctcctgatctttgctgcatccagtttgcaaagtggggtcccatcaaggttcagtggcagtggatctgggacagatttcactctcaccatcagcagtctgcaacctgaagattttgcaacttactactgtcaacagagttacagtacccctccgatcaccttcggccaagggacacgactggagattaaa

SEQ ID NO: 138 - protein, 108 aa, synthetic construct
  REGION 1..108: note = synthetic
DIQMTQSPSSLSASVGDRVTITCRASQSMSSYLNWYQQKPGRAPKLLIFAASSLQSGVPSRFSGSGSGTDFTLTISSLQPEDFATYYCQQSYSTPPITFGQGTRLEIK

SEQ ID NO: 139 - DNA, 18 bp, synthetic construct
  misc_feature 1..18: note = synthetic
  source 1..18: mol_type = other DNA
cagagcatgagcagctat

SEQ ID NO: 140 - protein, 6 aa, synthetic construct
  REGION 1..6: note = synthetic
QSMSSY

SEQ ID NO: 141-142 - skipped (2 entries)

SEQ ID NO: 143 - DNA, 30 bp, synthetic construct; identical to SEQ ID NO: 95
  misc_feature 1..30: note = synthetic
  source 1..30: mol_type = other DNA

SEQ ID NO: 144 - protein, 10 aa, synthetic construct
  REGION 1..10: note = synthetic
QQSYSTPPIT

SEQ ID NO: 145 - DNA, 354 bp, synthetic construct
  misc_feature 1..354: note = synthetic
  source 1..354: mol_type = other DNA
caggtccagctggtgcagtctggggctgaggtgaagatgcctgggtcctcggtgagggtctcctgcaaggcttctggaggcatcttcagcagttctactatcagttgggtgcgacaggcccctggacaagggcttgaatggatgggagagatcatccctgtctttggtacagtaaactacgcacagaagttccaggacagagtcatatttaccgcggacgaatctacgactacagcctacatggagctgagcagcctgaaatctggggacacggccgtatatttctgtgcgcgaaattggggattaggctctttttatatctggggccaagggacaatggtcaccgtctcttca

SEQ ID NO: 146 - protein, 118 aa, synthetic construct
  REGION 1..118: note = synthetic
QVQLVQSGAEVKMPGSSVRVSCKASGGIFSSSTISWVRQAPGQGLEWMGEIIPVFGTVNYAQKFQDRVIFTADESTTTAYMELSSLKSGDTAVYFCARNWGLGSFYIWGQGTMVTVSS

SEQ ID NO: 147 - DNA, 24 bp, synthetic construct
  misc_feature 1..24: note = synthetic
  source 1..24: mol_type = other DNA
ggaggcatcttcagcagttctact

SEQ ID NO: 148 - protein, 8 aa, synthetic construct
  REGION 1..8: note = synthetic
GGIFSSST

SEQ ID NO: 149 - DNA, 24 bp, synthetic construct
  misc_feature 1..24: note = synthetic
  source 1..24: mol_type = other DNA
atcatccctgtctttggtacagta

SEQ ID NO: 150 - protein, 8 aa, synthetic construct
  REGION 1..8: note = synthetic
IIPVFGTV

SEQ ID NO: 151 - DNA, 33 bp, synthetic construct
  misc_feature 1..33: note = synthetic
  source 1..33: mol_type = other DNA
gcgcgaaattggggattaggctctttttatatc

SEQ ID NO: 152 - protein, 11 aa, synthetic construct
  REGION 1..11: note = synthetic
ARNWGLGSFYI

SEQ ID NO: 153 - DNA, 324 bp, synthetic construct
  misc_feature 1..324: note = synthetic
  source 1..324: mol_type = other DNA
gaaattgtgttgacgcagtctccaggcaccctgtctttgtctccaggggaaagagccaccctctcctgcagggccagtcagagttttaacttcaactacttagcctggtaccagcagaaacctggccaggctcccagactcctcatctatggtgcatccagcagggccactggcatcccagacaggttcagtggcagtgggtctgggacagacttcactctcaccatcaacaggctggagcctgaagattttggagtgttttattgtcagcagtatgaaagcgcaccttggacgttcggccaagggaccaaggtggaaatcaaa

SEQ ID NO: 154 - protein, 108 aa, synthetic construct
  REGION 1..108: note = synthetic
EIVLTQSPGTLSLSPGERATLSCRASQSFNFNYLAWYQQKPGQAPRLLIYGASSRATGIPDRFSGSGSGTDFTLTINRLEPEDFGVFYCQQYESAPWTFGQGTKVEIK

SEQ ID NO: 155 - DNA, 21 bp, synthetic construct
  misc_feature 1..21: note = synthetic
  source 1..21: mol_type = other DNA
cagagttttaacttcaactac

SEQ ID NO: 156 - protein, 7 aa, synthetic construct
  REGION 1..7: note = synthetic
QSFNFNY

SEQ ID NO: 157-158 - skipped (2 entries)

SEQ ID NO: 159 - DNA, 27 bp, synthetic construct
  misc_feature 1..27: note = synthetic
  source 1..27: mol_type = other DNA
cagcagtatgaaagcgcaccttggacg

SEQ ID NO: 160 - protein, 9 aa, synthetic construct
  REGION 1..9: note = synthetic
QQYESAPWT

SEQ ID NO: 161 - DNA, 345 bp, synthetic construct
  misc_feature 1..345: note = synthetic
  source 1..345: mol_type = other DNA
gaggtgcagcttgtagagtctgggggagacttggtacatcctggcaggtccctgagactctcctgtgcagcctctggtttcccctttgatgagtatgccatgcactgggtccggcaagttccagggaagggcctggagtgggtctcaggtattagttggagtaataataacataggctatgcggactctgtgaagggccgattcaccatctccagagacaacgccaaaaactccctgtatctacaaatgaacagtctgagacctgaggacacggccttttattactgtgcaaaatctggaatctttgactcctggggccagggaaccctggtcaccgtctcctca

SEQ ID NO: 162 - protein, 115 aa, synthetic construct
  REGION 1..115: note = synthetic
EVQLVESGGDLVHPGRSLRLSCAASGFPFDEYAMHWVRQVPGKGLEWVSGISWSNNNIGYADSVKGRFTISRDNAKNSLYLQMNSLRPEDTAFYYCAKSGIFDSWGQGTLVTVSS

SEQ ID NO: 163 - DNA, 24 bp, synthetic construct
  misc_feature 1..24: note = synthetic
  source 1..24: mol_type = other DNA
ggtttcccctttgatgagtatgcc

SEQ ID NO: 164 - protein, 8 aa, synthetic construct
  REGION 1..8: note = synthetic
GFPFDEYA

SEQ ID NO: 165 - DNA, 24 bp, synthetic construct
  misc_feature 1..24: note = synthetic
  source 1..24: mol_type = other DNA
attagttggagtaataataacata

SEQ ID NO: 166 - protein, 8 aa, synthetic construct
  REGION 1..8: note = synthetic
ISWSNNNI

SEQ ID NO: 167 - DNA, 24 bp, synthetic construct
  misc_feature 1..24: note = synthetic
  source 1..24: mol_type = other DNA
gcaaaatctggaatctttgactcc

SEQ ID NO: 168 - protein, 8 aa, synthetic construct
  REGION 1..8: note = synthetic
AKSGIFDS

SEQ ID NO: 169 - DNA, 315 bp, synthetic construct
  misc_feature 1..315: note = synthetic
  source 1..315: mol_type = other DNA
gacatccagatgacccagtctccatcctccctgtctgcatctgtaggagacagagtcaccatcacttgccgggcaagtcagagcattagcagctatttaaattggtatcagcagaaaccagggaagctcctgatctatgctgcatccagtttgcaaagtggggtcccatcacggttcagtggcggtggatctgggacagatttcactctcaccatcagcagtctgcgacctgaagattttgcaacttactactgtcaacagagttactgtacccctccgatcaccttcggccaagggacacgactggagattaaa

SEQ ID NO: 170 - protein, 105 aa, synthetic construct
  REGION 1..105: note = synthetic
DIQMTQSPSSLSASVGDRVTITCRASQSISSYLNWYQQKPGKLLIYAASSLQSGVPSRFSGGGSGTDFTLTISSLRPEDFATYYCQQSYCTPPITFGQGTRLEIK

SEQ ID NO: 171 - DNA, 18 bp, synthetic construct
  misc_feature 1..18: note = synthetic
  source 1..18: mol_type = other DNA
cagagcattagcagctat

SEQ ID NO: 172 - protein, 6 aa, synthetic construct
  REGION 1..6: note = synthetic
QSISSY

SEQ ID NO: 173-174 - skipped (2 entries)

SEQ ID NO: 175 - DNA, 30 bp, synthetic construct
  misc_feature 1..30: note = synthetic
  source 1..30: mol_type = other DNA
caacagagttactgtacccctccgatcacc

SEQ ID NO: 176 - protein, 10 aa, synthetic construct
  REGION 1..10: note = synthetic
QQSYCTPPIT

SEQ ID NO: 177 - DNA, 354 bp, synthetic construct
  misc_feature 1..354: note = synthetic
  source 1..354: mol_type = other DNA
gaggtgcagctggtggagtccgggggaggcgtggtccagcctgggaggtccctgagactctcctgtgcagcctctggattcaccttcagtagttatggcatgcactgggtccgccaggctccaggcaagggactggagtgggtgacacttatatcatatgagggaaggaataaatactatgcagactccgtgaagggccgattcaccatttccagagacaattccaagaacacgctgtatctgcaaatgaacagcctgagagctgaggacacggctgtatattactgtgcgaaagataggaccctttacggtatggacgtctggggccaaggaaccacggtcaccgtctcctca

SEQ ID NO: 178 - protein, 118 aa, synthetic construct
  REGION 1..118: note = synthetic
EVQLVESGGGVVQPGRSLRLSCAASGFTFSSYGMHWVRQAPGKGLEWVTLISYEGRNKYYADSVKGRFTISRDNSKNTLYLQMNSLRAEDTAVYYCAKDRTLYGMDVWGQGTTVTVSS

SEQ ID NO: 179 - DNA, 24 bp, synthetic construct
  misc_feature 1..24: note = synthetic
  source 1..24: mol_type = other DNA
ggattcaccttcagtagttatggc

SEQ ID NO: 180 - protein, 8 aa, synthetic construct
  REGION 1..8: note = synthetic
GFTFSSYG

SEQ ID NO: 181 - DNA, 24 bp, synthetic construct
  misc_feature 1..24: note = synthetic
  source 1..24: mol_type = other DNA
atatcatatgagggaaggaataaa

SEQ ID NO: 182 - protein, 8 aa, synthetic construct
  REGION 1..8: note = synthetic
ISYEGRNK

SEQ ID NO: 183 - DNA, 33 bp, synthetic construct
  misc_feature 1..33: note = synthetic
  source 1..33: mol_type = other DNA
gcgaaagataggaccctttacggtatggacgtc

SEQ ID NO: 184 - protein, 11 aa, synthetic construct
  REGION 1..11: note = synthetic
AKDRTLYGMDV

SEQ ID NO: 185 - DNA, 363 bp, synthetic construct
  misc_feature 1..363: note = synthetic
  source 1..363: mol_type = other DNA
caggtcaccttgagggagtctggtcctgcgctggtgaaaaccacacagaccctcacactgacctgcaccttctctgggttctcactcagcactaatagaatgtgtgtgacctggatccgtcagcccccagggaaggccctggagtggcttgcgcgcattgattgggatggtgttaaatactacaacacatctctgaagaccaggctcaccatctccaaggacacctccaaaaaccaggtggtccttacaatgaccaacatggaccctgtggacacagccactttttactgtgcacggtcgacttcgttgactttttactactttgactactggggccagggaaccctggtcaccgtctcctca

SEQ ID NO: 186 - protein, 121 aa, synthetic construct
  REGION 1..121: note = synthetic
QVTLRESGPALVKTTQTLTLTCTFSGFSLSTNRMCVTWIRQPPGKALEWLARIDWDGVKYYNTSLKTRLTISKDTSKNQVVLTMTNMDPVDTATFYCARSTSLTFYYFDYWGQGTLVTVSS

SEQ ID NO: 187 - DNA, 30 bp, synthetic construct
  misc_feature 1..30: note = synthetic
  source 1..30: mol_type = other DNA
gggttctcactcagcactaatagaatgtgt

SEQ ID NO: 188 - protein, 10 aa, synthetic construct
  REGION 1..10: note = synthetic
GFSLSTNRMC

SEQ ID NO: 189 - DNA, 21 bp, synthetic construct
  misc_feature 1..21: note = synthetic
  source 1..21: mol_type = other DNA
attgattgggatggtgttaaa

SEQ ID NO: 190 - protein, 7 aa, synthetic construct
  REGION 1..7: note = synthetic
IDWDGVK

SEQ ID NO: 191 - DNA, 39 bp, synthetic construct
  misc_feature 1..39: note = synthetic
  source 1..39: mol_type = other DNA
gcacggtcgacttcgttgactttttactactttgactac

SEQ ID NO: 192 - protein, 13 aa, synthetic construct
  REGION 1..13: note = synthetic
ARSTSLTFYYFDY

SEQ ID NO: 193 - DNA, 324 bp, synthetic construct
  misc_feature 1..324: note = synthetic
  source 1..324: mol_type = other DNA
gacatccagatgacccagtctccatcctccctgtctgcatctgtaggagacagagtcaccatcacttgccgggcaagtcagagcattagcagctatttaaattggtatcagcagaaaccagggaaagcccctaagctcctgatctatgctgcatccagtttgcaaagtggggtcccatcaaggttcagtggcagtggatctgggacagatttcactctcaccatcagcagtctgcaacctgaagattttgcaacttactactgtcaacagagttacagtacccctccgatcaccttcggccaagggacacgactggagattaaa

SEQ ID NO: 194 - protein, 108 aa, synthetic construct
  REGION 1..108: note = synthetic
DIQMTQSPSSLSASVGDRVTITCRASQSISSYLNWYQQKPGKAPKLLIYAASSLQSGVPSRFSGSGSGTDFTLTISSLQPEDFATYYCQQSYSTPPITFGQGTRLEIK

SEQ ID NO: 195 - DNA, 18 bp, synthetic construct
  misc_feature 1..18: note = synthetic
  source 1..18: mol_type = other DNA
cagagcattagcagctat

SEQ ID NO: 196 - protein, 6 aa, synthetic construct
  REGION 1..6: note = synthetic
QSISSY

SEQ ID NO: 197-198 - skipped (2 entries)

SEQ ID NO: 199 - DNA, 30 bp, synthetic construct; identical to SEQ ID NO: 95
  misc_feature 1..30: note = synthetic
  source 1..30: mol_type = other DNA

SEQ ID NO: 200 - protein, 10 aa, synthetic construct
  REGION 1..10: note = synthetic
QQSYSTPPIT

SEQ ID NO: 201 - DNA, 345 bp, synthetic construct
  misc_feature 1..345: note = synthetic
  source 1..345: mol_type = other DNA
gaggtgcagctggtggagtctggaggaggcttggtccagccgggggggtccctgagactctcctgtgcagcctctgagttcaccgtcggtaccaaccacatgaactgggtccgccaggctccagggaagggactggagtgggtctcagttatttatagcggtggtaacacattctacgcagactccgtgaagggccgattcaccatctccagacacacttccaagaacacgctgtatcttcaaatgaacagcctgacagcagaggacacggccgtatattactgtgcgcgaggattggggggtatggacgtctggggccaagggaccacggtcaccgtctcctca

SEQ ID NO: 202 - protein, 115 aa, synthetic construct
  REGION 1..115: note = synthetic
EVQLVESGGGLVQPGGSLRLSCAASEFTVGTNHMNWVRQAPGKGLEWVSVIYSGGNTFYADSVKGRFTISRHTSKNTLYLQMNSLTAEDTAVYYCARGLGGMDVWGQGTTVTVSS

SEQ ID NO: 203 - DNA, 24 bp, synthetic construct
  misc_feature 1..24: note = synthetic
  source 1..24: mol_type = other DNA
gagttcaccgtcggtaccaaccac

SEQ ID NO: 204 - protein, 8 aa, synthetic construct
  REGION 1..8: note = synthetic
EFTVGTNH

SEQ ID NO: 205 - DNA, 21 bp, synthetic construct
  misc_feature 1..21: note = synthetic
  source 1..21: mol_type = other DNA
atttatagcggtggtaacaca

SEQ ID NO: 206 - protein, 7 aa, synthetic construct
  REGION 1..7: note = synthetic
IYSGGNT

SEQ ID NO: 207 - DNA, 27 bp, synthetic construct
  misc_feature 1..27: note = synthetic
  source 1..27: mol_type = other DNA
gcgcgaggattggggggtatggacgtc

SEQ ID NO: 208 - protein, 9 aa, synthetic construct
  REGION 1..9: note = synthetic
ARGLGGMDV

SEQ ID NO: 209 - DNA, 321 bp, synthetic construct
  misc_feature 1..321: note = synthetic
  source 1..321: mol_type = other DNA
gacatccagatgacccagtctccatcctccctgtctgcatctgtaggagacagagtcaccatcacttgccgggcgagtcaggtcattagcaattatttagcctggtatcagcagaaaccagggaaagttcctaggctcctgatctatgctgcatccactttgcaatcaggggtcccatctcgtttcagtggcagtggatctgggacagatttcactctcaccatcagcagcctgcagcctgaagatgttgcaacttattactgtcaaaagtataacagtgcccctcggacgttcggccaagggaccaaggtggaaatcaaa

SEQ ID NO: 210 - protein, 107 aa, synthetic construct
  REGION 1..107: note = synthetic
DIQMTQSPSSLSASVGDRVTITCRASQVISNYLAWYQQKPGKVPRLLIYAASTLQSGVPSRFSGSGSGTDFTLTISSLQPEDVATYYCQKYNSAPRTFGQGTKVEIK

SEQ ID NO: 211 - DNA, 18 bp, synthetic construct
  misc_feature 1..18: note = synthetic
  source 1..18: mol_type = other DNA
caggtcattagcaattat

SEQ ID NO: 212 - protein, 6 aa, synthetic construct
  REGION 1..6: note = synthetic
QVISNY

SEQ ID NO: 213-214 - skipped (2 entries)

SEQ ID NO: 215 - DNA, 27 bp, synthetic construct
  misc_feature 1..27: note = synthetic
  source 1..27: mol_type = other DNA
caaaagtataacagtgcccctcggacg

SEQ ID NO: 216 - protein, 9 aa, synthetic construct
  REGION 1..9: note = synthetic
QKYNSAPRT

SEQ ID NO: 217 - DNA, 360 bp, synthetic construct
  misc_feature 1..360: note = synthetic
  source 1..360: mol_type = other DNA
gaggtgcagctggtggagtctgggggaggcttggtccagcggggggagtccctgagactttactgtgcagcctctggattcacctttagtaaatattggatgaactgggtccgccaggctccagggaaggggctggagtgggtggccaacataaagggagatggaagtgagaaatactatgtggactctgtgaagggccggttcaccatctccagagacaacgccaagaactcactatatctacaaatgaacagcctgagagccgaggacacggctgtttattactgtgcgagagattattggggatcaggctactactttgacttctggggccagggaaccctggtcaccgtctcctca

SEQ ID NO: 218 - protein, 120 aa, synthetic construct
  REGION 1..120: note = synthetic
EVQLVESGGGLVQRGESLRLYCAASGFTFSKYWMNWVRQAPGKGLEWVANIKGDGSEKYYVDSVKGRFTISRDNAKNSLYLQMNSLRAEDTAVYYCARDYWGSGYYFDFWGQGTLVTVSS

SEQ ID NO: 219 - DNA, 24 bp, synthetic construct
  misc_feature 1..24: note = synthetic
  source 1..24: mol_type = other DNA
ggattcacctttagtaaatattgg

SEQ ID NO: 220 - protein, 8 aa, synthetic construct
  REGION 1..8: note = synthetic
GFTFSKYW

SEQ ID NO: 221 - DNA, 24 bp, synthetic construct
  misc_feature 1..24: note = synthetic
  source 1..24: mol_type = other DNA
ataaagggagatggaagtgagaaa

SEQ ID NO: 222 - protein, 8 aa, synthetic construct
  REGION 1..8: note = synthetic
IKGDGSEK

SEQ ID NO: 223 - DNA, 39 bp, synthetic construct
  misc_feature 1..39: note = synthetic
  source 1..39: mol_type = other DNA
gcgagagattattggggatcaggctactactttgacttc

SEQ ID NO: 224 - protein, 13 aa, synthetic construct
  REGION 1..13: note = synthetic
ARDYWGSGYYFDF

SEQ ID NO: 225 - DNA, 321 bp, synthetic construct
  misc_feature 1..321: note = synthetic
  source 1..321: mol_type = other DNA
gacatccagatgacccagtctccatcctccctgtctgcatctgtaggagacagagtcaccatcacttgccgggcaagtcagaacattaacaactatttaaattggtatcagcagaaaccagggaaagcccctaaactcctgatctatgctgcatccagtttccaaaatgcggtcccatcaaggttcagtggcagtggatctgggacagatttcactctcaccatcagcagtctgcaacctgaagattttgcaacttactactgtcaacagagttacaataccccgctcactttcggcggggggaccaaggtggagatcaaa

SEQ ID NO: 226 - protein, 107 aa, synthetic construct
  REGION 1..107: note = synthetic
DIQMTQSPSSLSASVGDRVTITCRASQNINNYLNWYQQKPGKAPKLLIYAASSFQNAVPSRFSGSGSGTDFTLTISSLQPEDFATYYCQQSYNTPLTFGGGTKVEIK

SEQ ID NO: 227 - DNA, 18 bp, synthetic construct
  misc_feature 1..18: note = synthetic
  source 1..18: mol_type = other DNA
cagaacattaacaactat

SEQ ID NO: 228 - protein, 6 aa, synthetic construct
  REGION 1..6: note = synthetic
QNINNY

SEQ ID NO: 229-230 - skipped (2 entries)

SEQ ID NO: 231 - DNA, 27 bp, synthetic construct
  misc_feature 1..27: note = synthetic
  source 1..27: mol_type = other DNA
caacagagttacaataccccgctcact

SEQ ID NO: 232 - protein, 9 aa, synthetic construct
  REGION 1..9: note = synthetic
QQSYNTPLT

SEQ ID NO: 233 - DNA, 390 bp, synthetic construct
  misc_feature 1..390: note = synthetic
  source 1..390: mol_type = other DNA
gaggtgcagctggtggagtctgggggaggcttggtccagtctggggggtccctgagactctcctgtgcagcctctggattcacctttagtagctattggatgagctgggtccgccaggctccagggaaggggctggagtgggtggccaacataaagcaagatggaagtgagaaatactatgtggactctgtgaagggccgattcaccatctccagagacaacgccaagaactcactgtatctgcaaatgaacagcctgagagccgatgacacggctgtgtattactgtgcgagagatgatattgtagtagtaccagctcctatgggatattactactactacttcggtatggacgtctggggccaagggaccacggtcaccgtctcctca

SEQ ID NO: 234 - protein, 130 aa, synthetic construct
  REGION 1..130: note = synthetic
EVQLVESGGGLVQSGGSLRLSCAASGFTFSSYWMSWVRQAPGKGLEWVANIKQDGSEKYYVDSVKGRFTISRDNAKNSLYLQMNSLRADDTAVYYCARDDIVVVPAPMGYYYYYFGMDVWGQGTTVTVSS

SEQ ID NO: 235 - DNA, 24 bp, synthetic construct
  misc_feature 1..24: note = synthetic
  source 1..24: mol_type = other DNA
ggattcacctttagtagctattgg

SEQ ID NO: 236 - protein, 8 aa, synthetic construct
  REGION 1..8: note = synthetic
GFTFSSYW

SEQ ID NO: 237 - DNA, 24 bp, synthetic construct
  misc_feature 1..24: note = synthetic
  source 1..24: mol_type = other DNA
ataaagcaagatggaagtgagaaa

SEQ ID NO: 238 - protein, 8 aa, synthetic construct
  REGION 1..8: note = synthetic
IKQDGSEK

SEQ ID NO: 239 - DNA, 69 bp, synthetic construct
  misc_feature 1..69: note = synthetic
  source 1..69: mol_type = other DNA
gcgagagatgatattgtagtagtaccagctcctatgggatattactactactacttcggtatggacgtc

SEQ ID NO: 240 - protein, 23 aa, synthetic construct
  REGION 1..23: note = synthetic
ARDDIVVVPAPMGYYYYYFGMDV

SEQ ID NO: 241 - DNA, 321 bp, synthetic construct
  misc_feature 1..321: note = synthetic
  source 1..321: mol_type = other DNA
gacatccagatgacccagtctccatcctccctgtctgcatctgtaggagacagagtcaccatcacttgccgggcaagtcagggcattagaaatgatttaggctggtatcagcagaaaccagggaaagcccctaagcgcctgatctatgctgcatccagtttgcaaagtggggtcccatcaaggttcagcggcagtggatctgggacagaattcactctcacaatcagcagcctgcagcctgaagattttgcaacttattactgtctacagcataatagttacccgtacacttttggccaggggaccaagctggagatcaaa

SEQ ID NO: 242 - protein, 107 aa, synthetic construct
  REGION 1..107: note = synthetic
DIQMTQSPSSLSASVGDRVTITCRASQGIRNDLGWYQQKPGKAPKRLIYAASSLQSGVPSRFSGSGSGTEFTLTISSLQPEDFATYYCLQHNSYPYTFGQGTKLEIK

SEQ ID NO: 243 - DNA, 18 bp, synthetic construct
  misc_feature 1..18: note = synthetic
  source 1..18: mol_type = other DNA
cagggcattagaaatgat

SEQ ID NO: 244 - protein, 6 aa, synthetic construct
  REGION 1..6: note = synthetic
QGIRND

SEQ ID NO: 245-246 - skipped (2 entries)

SEQ ID NO: 247 - DNA, 27 bp, synthetic construct
  misc_feature 1..27: note = synthetic
  source 1..27: mol_type = other DNA
ctacagcataatagttacccgtacact

SEQ ID NO: 248 - protein, 9 aa, synthetic construct
  REGION 1..9: note = synthetic
LQHNSYPYT

SEQ ID NO: 249 - DNA, 369 bp, synthetic construct
  misc_feature 1..369: note = synthetic
  source 1..369: mol_type = other DNA
gaagtgcagctggtggagtctgggggaggcttggttcagcctggcaggtccctgagactctcctgtgcagcctctggattcacctttgatgattttgccatgcactgggtccgacaagctccagggaagggcctggagtgggtctcaggtattagttggactggtggtaacatggactatgcgaactctgtgaagggccgattcaccatctccagagaggacgccaagaattccctgtatctgcaaatgaacagtctgagagctgcggacacggccttgtattactgtgtaaaagatataagggggatagtggctacggggggggcttttgatatctggggccgagggacaatggtcaccgtctcttca

SEQ ID NO: 250 - protein, 123 aa, synthetic construct
  REGION 1..123: note = synthetic
EVQLVESGGGLVQPGRSLRLSCAASGFTFDDFAMHWVRQAPGKGLEWVSGISWTGGNMDYANSVKGRFTISREDAKNSLYLQMNSLRAADTALYYCVKDIRGIVATGGAFDIWGRGTMVTVSS

SEQ ID NO: 251 - DNA, 24 bp, synthetic construct
  misc_feature 1..24: note = synthetic
  source 1..24: mol_type = other DNA
ggattcacctttgatgattttgcc

SEQ ID NO: 252 - protein, 8 aa, synthetic construct
  REGION 1..8: note = synthetic
GFTFDDFA

SEQ ID NO: 253 - DNA, 24 bp, synthetic construct
  misc_feature 1..24: note = synthetic
  source 1..24: mol_type = other DNA
attagttggactggtggtaacatg

SEQ ID NO: 254 - protein, 8 aa, synthetic construct
  REGION 1..8: note = synthetic
ISWTGGNM

SEQ ID NO: 255 - DNA, 48 bp, synthetic construct
  misc_feature 1..48: note = synthetic
  source 1..48: mol_type = other DNA
gtaaaagatataagggggatagtggctacggggggggcttttgatatc

SEQ ID NO: 256 - protein, 16 aa, synthetic construct
  REGION 1..16: note = synthetic
VKDIRGIVATGGAFDI

SEQ ID NO: 257 - DNA, 321 bp, synthetic construct
  misc_feature 1..321: note = synthetic
  source 1..321: mol_type = other DNA
gacatccagatgacccagtctccatcctccctgtctgcatctgtaggagacagagtcaccatctcttgccgggcaagtcagaccattagcacttatttaaattggtttcagcagaaaccagggaaagcccctaagctcctgatctatgttgtgtccagtttgcaaagtggggtcccatcaaggttcagtggcagtggatctgggacagatttcactctcaccatcagcagtctgcaacctgaagattttgcaacttattactgtcaacagagttacagtaccccattcactttcggccctgggaccaaagtggatatcaaa

SEQ ID NO: 258 - protein, 107 aa, synthetic construct
  REGION 1..107: note = synthetic
DIQMTQSPSSLSASVGDRVTISCRASQTISTYLNWFQQKPGKAPKLLIYVVSSLQSGVPSRFSGSGSGTDFTLTISSLQPEDFATYYCQQSYSTPFTFGPGTKVDIK

SEQ ID NO: 259 - DNA, 18 bp, synthetic construct
  misc_feature 1..18: note = synthetic
  source 1..18: mol_type = other DNA
cagaccattagcacttat

SEQ ID NO: 260 - protein, 6 aa, synthetic construct
  REGION 1..6: note = synthetic
QTISTY

SEQ ID NO: 261-262 - skipped (2 entries)

SEQ ID NO: 263 - DNA, 27 bp, synthetic construct
  misc_feature 1..27: note = synthetic
  source 1..27: mol_type = other DNA
caacagagttacagtaccccattcact

SEQ ID NO: 264 - protein, 9 aa, synthetic construct
  REGION 1..9: note = synthetic
QQSYSTPFT

SEQ ID NO: 265 - DNA, 345 bp, synthetic construct
  misc_feature 1..345: note = synthetic
  source 1..345: mol_type = other DNA
gaggtgcagctggtggagtctggaggaggcttggtccagccgggggggtccctgagactctcctgtgcagcctctggattcaccgtcggtaccaactacatgaactgggtccgccaggctccagggaagggactggagtggatctcagttatttatagcggtggtagcacattctacgcagactccgtgaagggccgattcaccatctccagacagacttcccagaacacgctgtatcttcaaatgaacagcctgagacctgaggacacggccgtatattactgtgcgagaggtatacgtggttttgatatctggggccaagggacaatggtcaccgtctcttca

SEQ ID NO: 266 - protein, 115 aa, synthetic construct
  REGION 1..115: note = synthetic
EVQLVESGGGLVQPGGSLRLSCAASGFTVGTNYMNWVRQAPGKGLEWISVIYSGGSTFYADSVKGRFTISRQTSQNTLYLQMNSLRPEDTAVYYCARGIRGFDIWGQGTMVTVSS

SEQ ID NO: 267 - DNA, 24 bp, synthetic construct
  misc_feature 1..24: note = synthetic
  source 1..24: mol_type = other DNA
ggattcaccgtcggtaccaactac

SEQ ID NO: 268 - protein, 8 aa, synthetic construct
  REGION 1..8: note = synthetic
GFTVGTNY

SEQ ID NO: 269 - DNA, 21 bp, synthetic construct
  misc_feature 1..21: note = synthetic
  source 1..21: mol_type = other DNA
atttatagcggtggtagcaca

SEQ ID NO: 270 - protein, 7 aa, synthetic construct
  REGION 1..7: note = synthetic
IYSGGST

SEQ ID NO: 271 - DNA, 27 bp, synthetic construct
  misc_feature 1..27: note = synthetic
  source 1..27: mol_type = other DNA
gcgagaggtatacgtggttttgatatc

SEQ ID NO: 272 - protein, 9 aa, synthetic construct
  REGION 1..9: note = synthetic
ARGIRGFDI

SEQ ID NO: 273 - DNA, 324 bp, synthetic construct
  misc_feature 1..324: note = synthetic
  source 1..324: mol_type = other DNA
gacatccagatgacccagtctccatcctccctgtctgcatctgtaggagacagagtcaccatcacttgccgggcaagtcagagcattagcagctatttaaattggtatcagcagaaaccagggaaagcccctaagctcctgatctatgctgcatccagtttgcaaagtggggtcccgtcaaggttcagtggcagtggatctgggacagatttcactctcaccatcagcagtctgcaacctgaagattttgcaacttactactgtcaacagagttacagtacccctccgatcaccttcggccaagggacacgactggagattaaa

SEQ ID NO: 274 - protein, 108 aa, synthetic construct; identical to SEQ ID NO: 194
  REGION 1..108: note = synthetic

SEQ ID NO: 275 - DNA, 18 bp, synthetic construct
  misc_feature 1..18: note = synthetic
  source 1..18: mol_type = other DNA
cagagcattagcagctat

SEQ ID NO: 276 - protein, 6 aa, synthetic construct
  REGION 1..6: note = synthetic
QSISSY

SEQ ID NO: 277-278 - skipped (2 entries)

SEQ ID NO: 279 - DNA, 30 bp, synthetic construct; identical to SEQ ID NO: 95
  misc_feature 1..30: note = synthetic
  source 1..30: mol_type = other DNA

SEQ ID NO: 280 - protein, 10 aa, synthetic construct
  REGION 1..10: note = synthetic
QQSYSTPPIT

SEQ ID NO: 281 - DNA, 345 bp, synthetic construct
  misc_feature 1..345: note = synthetic
  source 1..345: mol_type = other DNA
gaggtgcagctggtggagtctggaggaggcttggtccagccgggggggtccctgagactctcctgtgcagcctctgggtttaccatcagtaccaactacatgaactgggtccgccaggctccagggaaggggctggagtgggtcgcagttatttatagcagtggttccacatactatatcgactccgtgaagggccgattcaccatctccagactcacttccaagaacacggtgtatcttcaaatgagcagcctgaattctgaagacacggccgtgtattactgtgcgagggggatcaggggttttgatatttggggccaagggacaatggtcaccgtctcttca

SEQ ID NO: 282 - protein, 115 aa, synthetic construct
  REGION 1..115: note = synthetic
EVQLVESGGGLVQPGGSLRLSCAASGFTISTNYMNWVRQAPGKGLEWVAVIYSSGSTYYIDSVKGRFTISRLTSKNTVYLQMSSLNSEDTAVYYCARGIRGFDIWGQGTMVTVSS

SEQ ID NO: 283 - DNA, 24 bp, synthetic construct
  misc_feature 1..24: note = synthetic
  source 1..24: mol_type = other DNA
gggtttaccatcagtaccaactac

SEQ ID NO: 284 - protein, 8 aa, synthetic construct
  REGION 1..8: note = synthetic
GFTISTNY

SEQ ID NO: 285 - DNA, 21 bp, synthetic construct
  misc_feature 1..21: note = synthetic
  source 1..21: mol_type = other DNA
atttatagcagtggttccaca

SEQ ID NO: 286 - protein, 7 aa, synthetic construct
  REGION 1..7: note = synthetic
IYSSGST

SEQ ID NO: 287 - DNA, 27 bp, synthetic construct
  misc_feature 1..27: note = synthetic
  source 1..27: mol_type = other DNA
gcgagggggatcaggggttttgatatt

SEQ ID NO: 288 - protein, 9 aa, synthetic construct
  REGION 1..9: note = synthetic
ARGIRGFDI

SEQ ID NO: 289 - DNA, 372 bp, synthetic construct
  misc_feature 1..372: note = synthetic
  source 1..372: mol_type = other DNA
gaagtgcagctggtggagtcggggggaggcttggtacagcctggcaggtccctgagactctcctgtgcagcctctggattcaccattgatgatagtgccatgcactgggtccggcaaactccagggaagggcctggagtgggtctcaggtattagttggaaaagtggtagcataggttatgcggactctgtgaggggccgattcaccatctccagagacaacgccaagaattccctctatctgcaaatgaacagtctgagagttgaggacacggccttgtattactgtgtaaaagatataaggggcaactggaactacgggggaaactggttcgacccctggggccagggaaccctggtcactgtctcctca

SEQ ID NO: 290 - protein, 124 aa, synthetic construct
  REGION 1..124: note = synthetic
EVQLVESGGGLVQPGRSLRLSCAASGFTIDDSAMHWVRQTPGKGLEWVSGISWKSGSIGYADSVRGRFTISRDNAKNSLYLQMNSLRVEDTALYYCVKDIRGNWNYGGNWFDPWGQGTLVTVSS

SEQ ID NO: 291 - DNA, 24 bp, synthetic construct
  misc_feature 1..24: note = synthetic
  source 1..24: mol_type = other DNA
ggattcaccattgatgatagtgcc

SEQ ID NO: 292 - protein, 8 aa, synthetic construct
  REGION 1..8: note = synthetic
GFTIDDSA

SEQ ID NO: 293 - DNA, 24 bp, synthetic construct
  misc_feature 1..24: note = synthetic
  source 1..24: mol_type = other DNA
attagttggaaaagtggtagcata

SEQ ID NO: 294 - protein, 8 aa, synthetic construct
  REGION 1..8: note = synthetic
ISWKSGSI

SEQ ID NO: 295 - DNA, 51 bp, synthetic construct
  misc_feature 1..51: note = synthetic
  source 1..51: mol_type = other DNA
gtaaaagatataaggggcaactggaactacgggggaaactggttcgacccc

SEQ ID NO: 296 - protein, 17 aa, synthetic construct
  REGION 1..17: note = synthetic
VKDIRGNWNYGGNWFDP

SEQ ID NO: 297 - DNA, 345 bp, synthetic construct
  misc_feature 1..345: note = synthetic
  source 1..345: mol_type = other DNA
gaggtgcagctggtggagtctggaggaggcttggtccagcctggggggtccctgagactctcatgtgaagcctctgggttcaccgtcggtgtcaaccacatgaactgggtccgccaggctccagggaagggtctggagtgggtctcagttattttcagtagtggtaggacattctacggagactacgtgaaggggcgattaaccatcttcagacaaacctcccagaacacggtgtatcttcaaatgaatagcctgagaagtgaggacacggccatatattactgtgcgagagggattggcggtttggacatctggggccgagggacaatggtcaccgtctcttca

SEQ ID NO: 298 - protein, 115 aa, synthetic construct
  REGION 1..115: note = synthetic
EVQLVESGGGLVQPGGSLRLSCEASGFTVGVNHMNWVRQAPGKGLEWVSVIFSSGRTFYGDYVKGRLTIFRQTSQNTVYLQMNSLRSEDTAIYYCARGIGGLDIWGRGTMVTVSS

SEQ ID NO: 299 - DNA, 24 bp, synthetic construct
  misc_feature 1..24: note = synthetic
  source 1..24: mol_type = other DNA
gggttcaccgtcggtgtcaaccac

SEQ ID NO: 300 - protein, 8 aa, synthetic construct
  REGION 1..8: note = synthetic
GFTVGVNH

SEQ ID NO: 301 - DNA, 21 bp, synthetic construct
  misc_feature 1..21: note = synthetic
  source 1..21: mol_type = other DNA
attttcagtagtggtaggaca

SEQ ID NO: 302 - protein, 7 aa, synthetic construct
  REGION 1..7: note = synthetic
IFSSGRT

SEQ ID NO: 303 - DNA, 27 bp, synthetic construct
  misc_feature 1..27: note = synthetic
  source 1..27: mol_type = other DNA
gcgagagggattggcggtttggacatc

SEQ ID NO: 304 - protein, 9 aa, synthetic construct
  REGION 1..9: note = synthetic
ARGIGGLDI

SEQ ID NO: 305 - DNA, 369 bp, synthetic construct
  misc_feature 1..369: note = synthetic
  source 1..369: mol_type = other DNA
gaagtgcagctggtggagtctgggggaggcttggttcagcctggcaggtccctaagactctcctgtgcagcctctggattcacctttgatgattatgccttgcactgggtccggcaagctccagggaagggcctggagtgggtctcaggtattagttggactggtggtactatagactatgcggactctgtgaagggccgattcaccatctccagagacaacgccaagaactccctgtatctgcaaatgagcagtctgagaactgaggacacggccatatattactgtacaagagatatccgggggaactggaagtacggaggctggttcgacccctggggccagggaaccctggtcaccgtctcctca

SEQ ID NO: 306 - protein, 123 aa, synthetic construct
  REGION 1..123: note = synthetic
EVQLVESGGGLVQPGRSLRLSCAASGFTFDDYALHWVRQAPGKGLEWVSGISWTGGTIDYADSVKGRFTISRDNAKNSLYLQMSSLRTEDTAIYYCTRDIRGNWKYGGWFDPWGQGTLVTVSS

SEQ ID NO: 307 - DNA, 24 bp, synthetic construct
  misc_feature 1..24: note = synthetic
  source 1..24: mol_type = other DNA
ggattcacctttgatgattatgcc

SEQ ID NO: 308 - protein, 8 aa, synthetic construct
  REGION 1..8: note = synthetic
GFTFDDYA

SEQ ID NO: 309 - DNA, 24 bp, synthetic construct
  misc_feature 1..24: note = synthetic
  source 1..24: mol_type = other DNA
attagttggactggtggtactata

SEQ ID NO: 310 - protein, 8 aa, synthetic construct
  REGION 1..8: note = synthetic
ISWTGGTI

SEQ ID NO: 311 - DNA, 48 bp, synthetic construct
  misc_feature 1..48: note = synthetic
  source 1..48: mol_type = other DNA
acaagagatatccgggggaactggaagtacggaggctggttcgacccc

SEQ ID NO: 312 - protein, 16 aa, synthetic construct
  REGION 1..16: note = synthetic
TRDIRGNWKYGGWFDP

SEQ ID NO: 313 - DNA, 360 bp, synthetic construct
  misc_feature 1..360: note = synthetic
  source 1..360: mol_type = other DNA
caggtgcagctggtgcagtctgggactgaggtgaagaagcctggggcctcagtgaaggtctcctgcaaggcttctggatacaccttcaccgcctactatatgcactgggtgcgacaggcccctggtcaaggacttgactggatgggatggatcagccctaacagtggtttcacaaactatgcacagaagtttcagggcagggtcaccatgaccagggacacgtccatcaacacattttatatggagctgagtggactgagatctgacgacacggccgtatattactgtgcgcgagagggttctactcaccacaattctttcgacccctggggccagggaaccctggtcaccgtctcctca

SEQ ID NO: 314 - protein, 120 aa, synthetic construct
  REGION 1..120: note = synthetic
QVQLVQSGTEVKKPGASVKVSCKASGYTFTAYYMHWVRQAPGQGLDWMGWISPNSGFTNYAQKFQGRVTMTRDTSINTFYMELSGLRSDDTAVYYCAREGSTHHNSFDPWGQGTLVTVSS

SEQ ID NO: 315 - DNA, 24 bp, synthetic construct
  misc_feature 1..24: note = synthetic
  source 1..24: mol_type = other DNA
ggatacaccttcaccgcctactat

SEQ ID NO: 316 - protein, 8 aa, synthetic construct
  REGION 1..8: note = synthetic
GYTFTAYY

SEQ ID NO: 317 - DNA, 24 bp, synthetic construct
  misc_feature 1..24: note = synthetic
  source 1..24: mol_type = other DNA
atcagccctaacagtggtttcaca

SEQ ID NO: 318 - protein, 8 aa, synthetic construct
  REGION 1..8: note = synthetic
ISPNSGFT

SEQ ID NO: 319 - DNA, 39 bp, synthetic construct
  misc_feature 1..39: note = synthetic
  source 1..39: mol_type = other DNA
gcgcgagagggttctactcaccacaattctttcgacccc

SEQ ID NO: 320 - protein, 13 aa, synthetic construct
  REGION 1..13: note = synthetic
AREGSTHHNSFDP

SEQ ID NO: 321 - DNA, 342 bp, synthetic construct
  misc_feature 1..342: note = synthetic
  source 1..342: mol_type = other DNA
gaggtgcagctggtggagtctggaggaggcttggtccaaccgggggggtccctgaggctctcctgtgcagcctctgggttcaccgtcggtactaacttcatgaattgggtccgccaggctccagggaaggggctggagtgggtctcagcgatttatagcggtggtaccgctaactacgcagactccgtgaagggccgattcaccatttccagagacacttccaggaacacgctgtatcttcaaatgaacagcctgagaactgaggacacggccgtttattattgtgcgagaggggggggtatggacgtctggggccaagggaccacggtcaccgtctcctca

SEQ ID NO: 322 - protein, 114 aa, synthetic construct
  REGION 1..114: note = synthetic
EVQLVESGGGLVQPGGSLRLSCAASGFTVGTNFMNWVRQAPGKGLEWVSAIYSGGTANYADSVKGRFTISRDTSRNTLYLQMNSLRTEDTAVYYCARGGGMDVWGQGTTVTVSS

SEQ ID NO: 323 - DNA, 24 bp, synthetic construct
  misc_feature 1..24: note = synthetic
  source 1..24: mol_type = other DNA
gggttcaccgtcggtactaacttc

SEQ ID NO: 324 - protein, 8 aa, synthetic construct
  REGION 1..8: note = synthetic
GFTVGTNF

SEQ ID NO: 325 - DNA, 21 bp, synthetic construct
  misc_feature 1..21: note = synthetic
  source 1..21: mol_type = other DNA
atttatagcggtggtaccgct

SEQ ID NO: 326 - protein, 7 aa, synthetic construct
  REGION 1..7: note = synthetic
IYSGGTA

SEQ ID NO: 327 - DNA, 24 bp, synthetic construct
  misc_feature 1..24: note = synthetic
  source 1..24: mol_type = other DNA
gcgagaggggggggtatggacgtc

SEQ ID NO: 328 - protein, 8 aa, synthetic construct
  REGION 1..8: note = synthetic
ARGGGMDV

SEQ ID NO: 329 - DNA, 354 bp, synthetic construct
  misc_feature 1..354: note = synthetic
  source 1..354: mol_type = other DNA
caggtccagctggtgcagtctggggctgaggtgaagaagcctgggtcctcggtgaaggtctcctgcaaggcttctggaggcaccttcaacacctatgttctcagctgggtgcgacaggcccctggacaagggcttgagtggatgggagagatcatccctatcttaggtgcagcaaactacgcacagaacttccagggcagagtcacttttaccacggacgaatccacgaatacagcctacatggacctgagcagcctaagatctgaggacacggccgtgtattactgtgcgagagatcggacctccggggggttcgacccctggggccagggaaccctggtcactgtctcctca

SEQ ID NO: 330 - protein, 118 aa, synthetic construct
  REGION 1..118: note = synthetic
QVQLVQSGAEVKKPGSSVKVSCKASGGTFNTYVLSWVRQAPGQGLEWMGEIIPILGAANYAQNFQGRVTFTTDESTNTAYMDLSSLRSEDTAVYYCARDRTSGGFDPWGQGTLVTVSS

SEQ ID NO: 331 - DNA, 24 bp, synthetic construct
  misc_feature 1..24: note = synthetic
  source 1..24: mol_type = other DNA
ggaggcaccttcaacacctatgtt

SEQ ID NO: 332 - protein, 8 aa, synthetic construct
  REGION 1..8: note = synthetic
GGTFNTYV

SEQ ID NO: 333 - DNA, 24 bp, synthetic construct
  misc_feature 1..24: note = synthetic
  source 1..24: mol_type = other DNA
atcatccctatcttaggtgcagca

SEQ ID NO: 334 - protein, 8 aa, synthetic construct
  REGION 1..8: note = synthetic
IIPILGAA

SEQ ID NO: 335 - DNA, 33 bp, synthetic construct
  misc_feature 1..33: note = synthetic
  source 1..33: mol_type = other DNA
gcgagagatcggacctccggggggttcgacccc

SEQ ID NO: 336 - protein, 11 aa, synthetic construct
  REGION 1..11: note = synthetic
ARDRTSGGFDP

SEQ ID NO: 337 - DNA, 357 bp, synthetic construct
  misc_feature 1..357: note = synthetic
  source 1..357: mol_type = other DNA
caggttcagctggtgcagtctggagctgaggtggagaagcctggggcctcagtgaaggtctcctgcaaggcttctggttacatctttacccactatggtatcagctgggtgcgacaggcccctggacaaggacttgagtgggtgggctggatcagcccttacaatggttacacagactatgcacagaaactccagggcagagtcaccttgaccacagacacatccacgaccacagcctacatggagctgaggaacctgagatctgacgacacggccatgtattactgttcgagagggaggggcccttactggtccttcgatctctggggccgtggcaccctggtcaccgtctcctca

SEQ ID NO: 338 - protein, 119 aa, synthetic construct
  REGION 1..119: note = synthetic
QVQLVQSGAEVEKPGASVKVSCKASGYIFTHYGISWVRQAPGQGLEWVGWISPYNGYTDYAQKLQGRVTLTTDTSTTTAYMELRNLRSDDTAMYYCSRGRGPYWSFDLWGRGTLVTVSS

SEQ ID NO: 339 - DNA, 24 bp, synthetic construct
  misc_feature 1..24: note = synthetic
  source 1..24: mol_type = other DNA
ggttacatctttacccactatggt

SEQ ID NO: 340 - protein, 8 aa, synthetic construct
  REGION 1..8: note = synthetic
GYIFTHYG

SEQ ID NO: 341 - DNA, 24 bp, synthetic construct
  misc_feature 1..24: note = synthetic
  source 1..24: mol_type = other DNA
atcagcccttacaatggttacaca

SEQ ID NO: 342 - protein, 8 aa, synthetic construct
  REGION 1..8: note = synthetic
ISPYNGYT

SEQ ID NO: 343 - DNA, 36 bp, synthetic construct
  misc_feature 1..36: note = synthetic
  source 1..36: mol_type = other DNA
tcgagagggaggggcccttactggtccttcgatctc

SEQ ID NO: 344 - protein, 12 aa, synthetic construct
  REGION 1..12: note = synthetic
SRGRGPYWSFDL